European Patent Application EP 4 324 919 A2, published February 21, 2024. Title: Polypeptide variants. Applicant: Novozymes A/S. Application EP. The sequence listing filed with the application follows.

SEQUENCE LISTING (1 sequence)

SEQ ID NO: 1 - protein, 221 aa, Aspergillus oryzae
VPVNPEPDATSVENVALKTGSGDSQSDPIKADLEVKGQSALPFDVDCWAILCKGAPNVLQRVNEKTKNSNRDRSGANKGPFKDPQKWGIKALPPKNPSWSAQDFKSPEEYAFASSLQGGTNAILAPVNLASQNSQGGVLNGFYSANKVAQFDPSKPQQTKGTWFQITKFTGAAGPYCKALGSNDKSVCDKNKNIAGDWGFDPAKWAYQYDEKNNKFNYVGK